European Patent Specification EP 3 519 049 B1, published December 3, 2025. Title: SAFE AND EFFECTIVE METHOD OF TREATING PSORIASIS WITH ANTI-IL23 SPECIFIC ANTIBODY. Applicant: JANSSEN BIOTECH, INC. RANDAZZO, BRUCE WASFI, YASMINE. Application PCT/US2017/054217. The sequence listing filed with the application follows.

SEQUENCE LISTING (148 sequences)

SEQ ID NO: 1 - protein, 5 aa, Homo sapiens
NYAIS

SEQ ID NO: 2 - protein, 5 aa, Homo sapiens
SNYIS

SEQ ID NO: 3 - protein, 5 aa, Homo sapiens
NYWIS

SEQ ID NO: 4 - protein, 5 aa, Homo sapiens
SYWIT

SEQ ID NO: 5 - protein, 5 aa, Homo sapiens
NYWIG

SEQ ID NO: 6 - protein, 5 aa, Homo sapiens
SFGMS

SEQ ID NO: 7 - protein, 17 aa, Homo sapiens
GIIPMFGYANYAQKFQG

SEQ ID NO: 8 - protein, 17 aa, Homo sapiens
GIIPVFGFTHYAQKFQG

SEQ ID NO: 9 - protein, 17 aa, Homo sapiens
GIIPIFGHANYAQKFQG

SEQ ID NO: 10 - protein, 17 aa, Homo sapiens
IIIPPIGNAWYAQKFQG

SEQ ID NO: 11 - protein, 17 aa, Homo sapiens
LIDPNFGGAYYAQKFQG

SEQ ID NO: 12 - protein, 17 aa, Homo sapiens
LIDPVFGGAYYAQKFQG

SEQ ID NO: 13 - protein, 17 aa, Homo sapiens
LIDPMFGGAYYAQKFQG

SEQ ID NO: 14 - protein, 16 aa, Homo sapiens
INAHLGGTWYAQKFQG

SEQ ID NO: 15 - protein, 17 aa, Homo sapiens
ISPGTGINAYYAQKFQG

SEQ ID NO: 16 - protein, 17 aa, Artificial Sequence
  Synthesized human sequence
  unsure (1): Where Xaa can be G, I, or L
  unsure (2): Where Xaa can be I or S
  unsure (3): Where Xaa can be I, P, N, or D
  unsure (4): Where Xaa can be P, G, or A
  unsure (5): Where Xaa can be I, M, P,; T, H, N, or V
  unsure (6): Where Xaa can be F, I, G, or L
  unsure (7): Where Xaa can G or I
  unsure (8): Where Xaa can be H, Y, N, or G
  unsure (9): Where Xaa can be A or T
  unsure (10): Where Xaa can be N, W, or Y
XXXXXXXXXXYAQKFQG

SEQ ID NO: 17 - protein, 17 aa, Homo sapiens
WIRPGDSDTRYSPSFEG

SEQ ID NO: 18 - protein, 19 aa, Homo sapiens
VSYISSSGSSTYYADSVKG

SEQ ID NO: 19 - protein, 17 aa, Homo sapiens
IIDPSNSYTNYSPSFQG

SEQ ID NO: 20 - protein, 17 aa, Homo sapiens
IIDPSNSYTRYSPSFQG

SEQ ID NO: 21 - protein, 17 aa, Homo sapiens
IIDPSNSYTDYSPSFQG

SEQ ID NO: 22 - protein, 17 aa, Homo sapiens
IISPTGSVTWYSPSFQG

SEQ ID NO: 23 - protein, 17 aa, Homo sapiens
IISPTGSSTWYSPSFQG

SEQ ID NO: 24 - protein, 17 aa, Homo sapiens
FISPDGSHTWYSPSFQG

SEQ ID NO: 25 - protein, 17 aa, Homo sapiens
IISPSGSTTWYSPSFQG

SEQ ID NO: 26 - protein, 17 aa, Homo sapiens
IISPTGSATWYSPSFQG

SEQ ID NO: 27 - protein, 17 aa, Homo sapiens
IIDPVSSWTKYSPSFQG

SEQ ID NO: 28 - protein, 17 aa, Artificial Sequence
  Synthesized human sequence
  unsure (3): Where Xaa can be D or S
  unsure (5): Where Xaa can be S, V, D, or T
  unsure (6): Where Xaa can be N, S, or G
  unsure (8): Where Xaa can be Y, W, T, H, V, S, or A
  unsure (10): Where Xaa can be N, D, R, K, or W
IIXPXXSXTXYSPSFQG

SEQ ID NO: 29 - protein, 17 aa, Homo sapiens
NISSSGSSTYYADSVKG

SEQ ID NO: 30 - protein, 19 aa, Homo sapiens
NIEHKYLNYATYYAASVKG

SEQ ID NO: 31 - protein, 19 aa, Homo sapiens
NIEHKFMGYTTYYAAGVKG

SEQ ID NO: 32 - protein, 19 aa, Homo sapiens
GIEHKYLSYTTHYAASVKG

SEQ ID NO: 33 - protein, 19 aa, Homo sapiens
SIEHKYTGYTTYYAAPVKG

SEQ ID NO: 34 - protein, 19 aa, Homo sapiens
QIEHKYLSYTTLYAASVKG

SEQ ID NO: 35 - protein, 19 aa, Homo sapiens
SIEHKYLSYTTFYAASVKG

SEQ ID NO: 36 - protein, 19 aa, Homo sapiens
NIEGKYTSYTTYYAASVKG

SEQ ID NO: 37 - protein, 19 aa, Homo sapiens
GIEHKYLSYATLYAASVKG

SEQ ID NO: 38 - protein, 19 aa, Homo sapiens
NIEHKYLGYATVYAASVKG

SEQ ID NO: 39 - protein, 19 aa, Homo sapiens
SIEHKYLSYATYYAAGVKG

SEQ ID NO: 40 - protein, 8 aa, Homo sapiens
DIYAGMDV

SEQ ID NO: 41 - protein, 18 aa, Homo sapiens
SKKGMYGGWTYPLMMFDL

SEQ ID NO: 42 - protein, 7 aa, Homo sapiens
HYYGMDY

SEQ ID NO: 43 - protein, 12 aa, Homo sapiens
GTFWSFGNYFAN

SEQ ID NO: 44 - protein, 8 aa, Homo sapiens
WYYKPFDV

SEQ ID NO: 45 - protein, 12 aa, Homo sapiens
YWGTPYLMQFDN

SEQ ID NO: 46 - protein, 12 aa, Homo sapiens
RASQSVLGNYLA

SEQ ID NO: 47 - protein, 12 aa, Homo sapiens
RASQSVSSNYLA

SEQ ID NO: 48 - protein, 13 aa, Homo sapiens
SGSSSNIGSYYVN

SEQ ID NO: 49 - protein, 11 aa, Homo sapiens
RASQSIFYNLA

SEQ ID NO: 50 - protein, 14 aa, Homo sapiens
TGSSSNIGSGYDVH

SEQ ID NO: 51 - protein, 14 aa, Homo sapiens
TGTSSDVGGYNSVS

SEQ ID NO: 52 - protein, 7 aa, Homo sapiens
GASSRAT

SEQ ID NO: 53 - protein, 7 aa, Homo sapiens
YASRRAT

SEQ ID NO: 54 - protein, 7 aa, Homo sapiens
GNTHRPS

SEQ ID NO: 55 - protein, 7 aa, Homo sapiens
GASNRAT

SEQ ID NO: 56 - protein, 7 aa, Homo sapiens
GNSKRPS

SEQ ID NO: 57 - protein, 7 aa, Homo sapiens
SVSSRPS

SEQ ID NO: 58 - protein, 9 aa, Homo sapiens
HQYGSISTT

SEQ ID NO: 59 - protein, 9 aa, Homo sapiens
QQYSHLLIT

SEQ ID NO: 60 - protein, 9 aa, Homo sapiens
QQYSHISLT

SEQ ID NO: 61 - protein, 9 aa, Homo sapiens
QQFAHILLT

SEQ ID NO: 62 - protein, 9 aa, Homo sapiens
QQTSNTPFT

SEQ ID NO: 63 - protein, 9 aa, Homo sapiens
QQFITYLPT

SEQ ID NO: 64 - protein, 9 aa, Homo sapiens
QQDALSPFT

SEQ ID NO: 65 - protein, 9 aa, Homo sapiens
QQDRGTPFT

SEQ ID NO: 66 - protein, 9 aa, Homo sapiens
QQSLNIPFT

SEQ ID NO: 67 - protein, 9 aa, Homo sapiens
QQDTSSPFT

SEQ ID NO: 68 - protein, 10 aa, Artificial Sequence
  Synthesized human sequence
  unsure (3): Where Xaa can be T, F, D, or S
  unsure (4): Where Xaa can be S, I, A, T, R, or L
  unsure (5): Where Xaa can be N, T, L, S, or G
  unsure (6): Where Xaa can be T, Y, S, or I
  unsure (7): Where Xaa can be P or L
  unsure (8): Where Xaa can be F or P
QQXXXXXXFT

SEQ ID NO: 69 - protein, 11 aa, Homo sapiens
QTYASLGPGEV

SEQ ID NO: 70 - protein, 9 aa, Homo sapiens
QQYSSEPVT

SEQ ID NO: 71 - protein, 9 aa, Homo sapiens
SSWTPSSVV

SEQ ID NO: 72 - protein, 11 aa, Homo sapiens
SSWTDTPNMIV

SEQ ID NO: 73 - protein, 11 aa, Homo sapiens
ASWTDGLSLVV

SEQ ID NO: 74 - protein, 11 aa, Artificial Sequence
  Synthesized human sequence
  unsure (1): Where Xaa can be S or A
  unsure (6): Where Xaa can be T or G
  unsure (7): Where Xaa can be P or L
  unsure (8): Where Xaa can be S or N
  unsure (9): Where Xaa can be S, M, or L
  unsure (10): Where Xaa can be I or V
XSWTDXXXXXV

SEQ ID NO: 75 - protein, 11 aa, Homo sapiens
SSYDTNKPLVV

SEQ ID NO: 76 - protein, 11 aa, Homo sapiens
GSYDVYGRFYV

SEQ ID NO: 77 - protein, 11 aa, Homo sapiens
SSYYFYLQRIV

SEQ ID NO: 78 - protein, 11 aa, Homo sapiens
QTYYFSYSGPV

SEQ ID NO: 79 - protein, 11 aa, Homo sapiens
GSWDPIFSYEV

SEQ ID NO: 80 - protein, 117 aa, Homo sapiens
QVQLVQSGAEVKKPGSSVKVSCKASGGTFSNYAISWVRQAPGQGLEWMGGIIPMFGYANYAQKFQGRVTITADESTSTAYMELSSLRSEDTAVYYCARDIYAGMDVWGQGTLVTVSS

SEQ ID NO: 81 - protein, 117 aa, Homo sapiens
QVQLVQSGAEVKKPGSSVKVSCKASGGTFSNYAISWVRQAPGQGLEWMGGIIPVFGFTHYAQKFQGRVTITADESTSTAYMELSSLRSEDTAVYYCARDIYAGMDVWGQGTLVTVSS

SEQ ID NO: 82 - protein, 108 aa, Homo sapiens
DIVLTQSPATLSLSPGERATLSCRASQSVLGNYLAWYQQKPGQAPRLLIYGASSRATGVPARFSGSGSGTDFTLTISSLEPEDFAVYYCHQYGSISTTFGQGTKVEIK

SEQ ID NO: 83 - protein, 108 aa, Homo sapiens
DIVLTQSPATLSLSPGERATLSCRASQSVLGNYLAWYQQKPGQAPRLLIYGASSRATGVPARFSGSGSGTDFTLTISSLEPEDFAVYYCQQYSHISLTFGQGTKVEIK

SEQ ID NO: 84 - protein, 108 aa, Homo sapiens
DIVLTQSPATLSLSPGERATLSCRASQSVLGNYLAWYQQKPGQAPRLLIYGASSRATGVPARFSGSGSGTDFTLTISSLEPEDFAVYYCQQYSHLIITFGQGTKVEIK

SEQ ID NO: 85 - protein, 108 aa, Homo sapiens
DIVLTQSPATLSLSPGERATLSCRASQSVLGNYLAWYQQKPGQAPRLLIYGASSRATGVPARFSGSGSGTDFTLTISSLEPEDFAVYYCQQFAHILLTFGQGTKVEIK

SEQ ID NO: 86 - protein, 127 aa, Homo sapiens
QVQLVQSGAEVKKPGSSVKVSCKASGGTFSSNYISWVRQAPGQGLEWMGGIIPIFGHANYAQKFQGRVTITADESTSTAYMELSSLRSEDTAVYYCARSKKGMYGGWTYPLMMFDLWGQGTLVTVSS

SEQ ID NO: 87 - protein, 127 aa, Homo sapiens
QVQLVQSGAEVKKPGSSVKVSCKASGGTFSSNYISWVRQAPGQGLEWMGIIIPPIGNAWYAQKFQGRVTITADESTSTAYMELSSLRSEDTAVYYCARSKKGMYGGWTYPLMMFDLWGQGTLVTVSS

SEQ ID NO: 88 - protein, 127 aa, Homo sapiens
QVQLVQSGAEVKKPGSSVKVSCKASGGTFSSNYISWVRQAPGQGLEWMGISPGTGINAYYAQKFQGRVTITADESTSTAYMELSSLRSEDTAVYYCARSKKGMYGGWTYPLMMFDLWGQGTLVTVSS

SEQ ID NO: 89 - protein, 126 aa, Homo sapiens
QVQLVQSGAEVKKPGSSVKVSCKASGGTFSSNYISWVRQAPGQGLEWMGINAHLGGTWYAQKFQGRVTITADESTSTAYMELSSLRSEDTAVYYCARSKKGMYGGWTYPLMMFDLWGQGTLVTVSS

SEQ ID NO: 90 - protein, 127 aa, Homo sapiens
QVQLVQSGAEVKKPGSSVKVSCKASGGTFSSNYISWVRQAPGQGLEWMGLIDPNFGGAYYAQKFQGRVTITADESTSTAYMELSSLRSEDTAVYYCARSKKGMYGGWTYPLMMFDLWGQGTLVTVSS

SEQ ID NO: 91 - protein, 127 aa, Homo sapiens
QVQLVQSGAEVKKPGSSVKVSCKASGGTFSSNYISWVRQAPGQGLEWMGLIDPVFGGAYYAQKFQGRVTITADESTSTAYMELSSLRSEDTAVYYCARSKKGMYGGWTYPLMMFDLWGQGTLVTVSS

SEQ ID NO: 92 - protein, 127 aa, Homo sapiens
QVQLVQSGAEVKKPGSSVKVSCKASGGTFSSNYISWVRQAPGQGLEWMGLIDPMFGGAYYAQKFQGRVTITADESTSTAYMELSSLRSEDTAVYYCARSKKGMYGGWTYPLMMFDLWGQGTLVTVSS

SEQ ID NO: 93 - protein, 108 aa, Homo sapiens
DIVLTQSPATLSLSPGERATLSCRASQSVSSNYLAWYQQKPGQAPRLLIYYASRRATGVPARFSGSGSGTDFTLTISSLEPEDFATYYCQQTSNTPFTFGQGTKVEIK

SEQ ID NO: 94 - protein, 108 aa, Homo sapiens
EIVLTQSPATLSLSPGERATLSCRASQSVSSNYLAWYQQKPGQAPRLLIYYASRRATGVPARFSGSGSGTDFTLTISSLEPEDFAVYYCQQTSNTPFTFGQGTKVEIK

SEQ ID NO: 95 - protein, 108 aa, Homo sapiens
DIVLTQSPATLSLSPGERATLSCRASQSVSSNYLAWYQQKPGQAPRLLIYYASRRATGVPARFSGSGSGTDFTLTISSLEPEDFAVYYCQQFITYLPTFGQGTKVEIK

SEQ ID NO: 96 - protein, 108 aa, Homo sapiens
DIVLTQSPATLSLSPGERATLSCRASQSVSSNYLAWYQQKPGQAPRLLIYYASRRATGVPARFSGSGSGTDFTLTISSLEPEDFAVYYCQQDALSPFTFGQGTKVEIK

SEQ ID NO: 97 - protein, 108 aa, Homo sapiens
DIVLTQSPATLSLSPGERATLSCRASQSVSSNYLAWYQQKPGQAPRLLIYYASRRATGVPARFSGSGSGTDFTLTISSLEPEDFAVYYCQQDRGTPFTFGQGTKVEIK

SEQ ID NO: 98 - protein, 108 aa, Homo sapiens
DIVLTQSPATLSLSPGERATLSCRASQSVSSNYLAWYQQKPGQAPRLLIYYASRRATGVPARFSGSGSGTDFTLTISSLEPEDFAVYYCQQSLNIPFTFGQGTKVEIK

SEQ ID NO: 99 - protein, 116 aa, Homo sapiens
QVQLVQSGAEVKKPGESLKISCKGSGYSFTNYWISWVRQAPGKGLEWMGWIRPGDSDTRYSPSFEGQVTISADKSISTAYLQWSSLKASDTAMYYCARHYYGMDYWGQGTLVTVSS

SEQ ID NO: 100 - protein, 110 aa, Homo sapiens
DIVLTQPPSVSGAPGQRVTISCSGSSSNIGSYYVNWYQQLPGTAPKLLIYGNTHRPSGVPDRFSGSKSGTSASLAITGLQSEDEADYYCQTYASLGPGEVFGGGTKLTVL

SEQ ID NO: 101 - protein, 121 aa, Homo sapiens
QVQLVESGGGLVQPGGSLRLSCAASGFTFSSYWITWVRQAPGKGLEWVSYISSSGSSTYYADSVKGRFTISRDNSKNTLYLQMNSLRAEDTAVYYCARGTFWSFGNYFANWGQGTLVTVSS

SEQ ID NO: 102 - protein, 107 aa, Homo sapiens
DIVLTQSPATLSLSPGERATLSCRASQSIFYNLAWYQQKPGQAPRLLIYGASNRATGVPARFSGSGSGTDFTLTISSLEPEDFATYYCQQYSSEPVTFGQGTKVEIK

SEQ ID NO: 103 - protein, 117 aa, Homo sapiens
QVQLVQSGAEVKKPGESLKISCKGSGYSFSNYWIGWVRQMPGKGLEWMGIIDPSNSYTNYSPSFQGQVTISADKSISTAYLQWSSLKASDTAMYYCARWYYKPFDVWGQGTLVTVSS

SEQ ID NO: 104 - protein, 117 aa, Homo sapiens
QVQLVQSGAEVKKPGESLKISCKGSGYSFSNYWIGWVRQMPGKGLEWMGIIDPSNSYTDYSPSFQGQVTISADKSISTAYLQWSSLKASDTAMYYCARWYYKPFDVWGQGTLVTVSS

SEQ ID NO: 105 - protein, 117 aa, Homo sapiens
QVQLVQSGAEVKKPGESLKISCKGSGYSFSNYWIGWVRQMPGKGLEWMGIIDPSNSYTRYSPSFQGQVTISADKSISTAYLQWSSLKASDTAMYYCARWYYKPFDVWGQGTLVTVSS

SEQ ID NO: 106 - protein, 117 aa, Homo sapiens
EVQLVQSGAEVKKPGESLKISCKGSGYSFSNYWIGWVRQMPGKGLEWMGIIDPSNSYTRYSPSFQGQVTISADKSISTAYLQWSSLKASDTAMYYCARWYYKPFDVWGQGTLVTVSS

SEQ ID NO: 107 - protein, 117 aa, Homo sapiens
QVQLVQSGAEVKKPGESLKISCKGSGYSFSNYWIGWVRQMPGKGLEWMGIIDPVSSWTKYSPSFQGQVTISADKSISTAYLQWSSLKASDTAMYYCARWYYKPFDVWGQGTLVTVSS

SEQ ID NO: 108 - protein, 117 aa, Homo sapiens
QVQLVQSGAEVKKPGESLKISCKGSGYSFSNYWIGWVRQMPGKGLEWMGIISPSGSTTWYSPSFQGQVTISADKSISTAYLQWSSLKASDTAMYYCARWYYKPFDVWGQGTLVTVSS

SEQ ID NO: 109 - protein, 117 aa, Homo sapiens
QVQLVQSGAEVKKPGESLKISCKGSGYSFSNYWIGWVRQMPGKGLEWMGFISPDGSHTWYSPSFQGQVTISADKSISTAYLQWSSLKASDTAMYYCARWYYKPFDVWGQGTLVTVSS

SEQ ID NO: 110 - protein, 117 aa, Homo sapiens
QVQLVQSGAEVKKPGESLKISCKGSGYSFSNYWIGWVRQMPGKGLEWMGIISPTGSVTWYSPSFQGQVTISADKSISTAYLQWSSLKASDTAMYYCARWYYKPFDVWGQGTLVTVSS

SEQ ID NO: 111 - protein, 117 aa, Homo sapiens
QVQLVQSGAEVKKPGESLKISCKGSGYSFSNYWIGWVRQMPGKGLEWMGIISPTGSSTWYSPSFQGQVTISADKSISTAYLQWSSLKASDTAMYYCARWYYKPFDVWGQGTLVTVSS

SEQ ID NO: 112 - protein, 117 aa, Homo sapiens
QVQLVQSGAEVKKPGESLKISCKGSGYSFSNYWIGWVRQMPGKGLEWMGIISPTGSATWYSPSFQGQVTISADKSISTAYLQWSSLKASDTAMYYCARWYYKPFDVWGQGTLVTVSS

SEQ ID NO: 113 - protein, 109 aa, Homo sapiens
DIVLTQPPSVSGAPGQRVTISCTGSSSNIGSGYDVHWYQQLPGTAPKLLIYGNSKRPSGVPDRFSGSKSGTSASLAITGLQSEDEADYYCSSWTPSSVVFGGGTKLTVL

SEQ ID NO: 114 - protein, 111 aa, Homo sapiens
DIVLTQPPSVSGAPGQRVTISCTGSSSNIGSGYDVHWYQQLPGTAPKLLIYGNSKRPSGVPDRFSGSKSGTSASLAITGLQSEDEADYYCSSWTDTPNMIVFGGGTKLTVL

SEQ ID NO: 115 - protein, 111 aa, Homo sapiens
DIVLTQPPSVSGAPGQRVTISCTGSSSNIGSGYDVHWYQQLPGTAPKLLIYGNSKRPSGVPDRFSGSKSGTSASLAITGLQSEDEADYYCASWTDGLSLVVFGGGTKLTVL

SEQ ID NO: 116 - protein, 111 aa, Homo sapiens
QSVLTQPPSVSGAPGQRVTISCTGSSSNIGSGYDVHWYQQLPGTAPKLLIYGNSKRPSGVPDRFSGSKSGTSASLAITGLQSEDEADYYCASWTDGLSLVVFGGGTKLTVL

SEQ ID NO: 117 - protein, 121 aa, Homo sapiens
QVQLVESGGGLVQPGGSLRLSCAASGFTFSSFGMSWVRQAPGKGLEWVSNISSSGSSTYYADSVKGRFTISRDNSKNTLYLQMNSLRAEDTAVYYCARYWGTPYLMQFDNWGQGTLVTVSS

SEQ ID NO: 118 - protein, 123 aa, Homo sapiens
QVQLVESGGGLVQPGGSLRLSCAASGFTFSSFGMSWVRQAPGKGLEWVSNIEHKFMGYTTYYAAGVKGRFTISRDNSKNTLYLQMNSLRAEDTAVYYCARYWGTPYLMQFDNWGQGTLVTVSS

SEQ ID NO: 119 - protein, 123 aa, Homo sapiens
QVQLVESGGGLVQPGGSLRLSCAASGFTFSSFGMSWVRQAPGKGLEWVSSIEHKYTGYTTYYAAPVKGRFTISRDNSKNTLYLQMNSLRAEDTAVYYCARYWGTPYLMQFDNWGQGTLVTVSS

SEQ ID NO: 120 - protein, 123 aa, Homo sapiens
QVQLVESGGGLVQPGGSLRLSCAASGFTFSSFGMSWVRQAPGKGLEWVSNIEHKYTSYTTYYAASVKGRFTISRDNSKNTLYLQMNSLRAEDTAVYYCARYWGTPYLMQFDNWGQGTLVTVSS

SEQ ID NO: 121 - protein, 123 aa, Homo sapiens
QVQLVESGGGLVQPGGSLRLSCAASGFTFSSFGMSWVRQAPGKGLEWVSNIEHKYLNYATYYAASVKGRFTISRDNSKNTLYLQMNSLRAEDTAVYYCARYWGTPYLMQFDNWGQGTLVTVSS

SEQ ID NO: 122 - protein, 123 aa, Homo sapiens
QVQLVESGGGLVQPGGSLRLSCAASGFTFSSFGMSWVRQAPGKGLEWVSNIEHKYLGYATVYAASVKGRFTISRDNSKNTLYLQMNSLRAEDTAVYYCARYWGTPYLMQFDNWGQGTLVTVSS

SEQ ID NO: 123 - protein, 123 aa, Homo sapiens
QVQLVESGGGLVQPGGSLRLSCAASGFTFSSFGMSWVRQAPGKGLEWVSSIEHKYLSYATYYAAGVKGRFTISRDNSKNTLYLQMNSLRAEDTAVYYCARYWGTPYLMQFDNWGQGTLVTVSS

SEQ ID NO: 124 - protein, 123 aa, Homo sapiens
QVQLVESGGGLVQPGGSLRLSCAASGFTFSSFGMSWVRQAPGKGLEWVSSIEHKYLSYTTFYAASVKGRFTISRDNSKNTLYLQMNSLRAEDTAVYYCARYWGTPYLMQFDNWGQGTLVTVSS

SEQ ID NO: 125 - protein, 123 aa, Homo sapiens
QVQLVESGGGLVQPGGSLRLSCAASGFTFSSFGMSWVRQAPGKGLEWVSGIEHKYLSYTTHYAASVKGRFTISRDNSKNTLYLQMNSLRAEDTAVYYCARYWGTPYLMQFDNWGQGTLVTVSS

SEQ ID NO: 126 - protein, 123 aa, Homo sapiens
QVQLVESGGGLVQPGGSLRLSCAASGFTFSSFGMSWVRQAPGKGLEWVSQIEHKYLSYTTLYAASVKGRFTISRDNSKNTLYLQMNSLRAEDTAVYYCARYWGTPYLMQFDNWGQGTLVTVSS

SEQ ID NO: 127 - protein, 123 aa, Homo sapiens
QVQLVESGGGLVQPGGSLRLSCAASGFTFSSFGMSWVRQAPGKGLEWVSGIEHKYLSYATLYAASVKGRFTISRDNSKNTLYLQMNSLRAEDTAVYYCARYWGTPYLMQFDNWGQGTLVTVSS

SEQ ID NO: 128 - protein, 111 aa, Homo sapiens
DIALTQPASVSGSPGQSITISCTGTSSDVGGYNSVSWYQQHPGKAPKLMIYSVSSRPSGVSNRFSGSKSGNTASLTISGLQAEDEADYYCSSYDTNKPLVVFGGGTKLTVL

SEQ ID NO: 129 - protein, 111 aa, Homo sapiens
DIALTQPASVSGSPGQSITISCTGTSSDVGGYNSVSWYQQHPGKAPKLMIYSVSSRPSGVSNRFSGSKSGNTASLTISGLQAEDEADYYCSSYYFYLQRIVFGGGTKLTVL

SEQ ID NO: 130 - protein, 111 aa, Homo sapiens
DIALTQPASVSGSPGQSITISCTGTSSDVGGYNSVSWYQQHPGKAPKLMIYSVSSRPSGVSNRFSGSKSGNTASLTISGLQAEDEADYYCQTYYFSYSGPVFGGGTKLTVL

SEQ ID NO: 131 - protein, 111 aa, Homo sapiens
DIALTQPASVSGSPGQSITISCTGTSSDVGGYNSVSWYQQHPGKAPKLMIYSVSSRPSGVSNRFSGSKSGNTASLTISGLQAEDEADYYCGSYDVYGRFYVFGGGTKLTVL

SEQ ID NO: 132 - protein, 111 aa, Homo sapiens
DIALTQPASVSGSPGQSITISCTGTSSDVGGYNSVSWYQQHPGKAPKLMIYSVSSRPSGVSNRFSGSKSGNTASLTISGLQAEDEADYYCGSWDPIFSYEVFGGGTKLTVL

SEQ ID NO: 133 - DNA, 381 bp, Homo sapiens
caggtgcagctggtgcagtctggggctgaggtgaagaagcctgggtcctcggtgaaggtctcctgcaaggcttctggaggcaccttcagcagcaactacatcagctgggtgcgacaggcccctggacaagggcttgagtggatggggatcagccctggcaccggtatcaacgcatactacgcacagaagttccagggcagagtcacgattaccgcggacgaatccacgagcacagcctacatggagctgagcagcctgagatctgaggacacggccgtgtattactgtgcgagaagcaagaagggcatgtacggcggctggacctaccccctgatgatgttcgacctgtggggccagggcaccctggtgaccgtgagcagc

SEQ ID NO: 134 - DNA, 381 bp, Homo sapiens
caggtgcagctggtgcagagcggcgccgaggtgaagaagcccggcagcagcgtgaaggtgagctgcaaggccagcggcggcaccttcagcagcaactacatcagctgggtgcgccaggcccccggccagggcctggagtggatgggcatcagccccggcaccggcatcaacgcctactacgcccagaagttccagggccgcgtgaccatcaccgccgacgagagcaccagcaccgcctacatggagctgagcagcctgcgcagcgaggacaccgccgtgtactactgcgcccgcagcaagaagggcatgtacggcggctggacctaccccctgatgatgttcgacctgtggggccagggcaccctggtgaccgtgagcagc

SEQ ID NO: 135 - DNA, 381 bp, Homo sapiens
caggtgcaattggttcagtctggcgcggaagtgaaaaaaccgggcagcagcgtgaaagtgagctgcaaagcctccggaggcactttttcttctaattatatttcttgggtgcgccaagcccctgggcagggtctcgagtggatgggcatttctcctggtactggtattaatgcttattatgctcagaagtttcagggtcgggtgaccattaccgcggatgaaagcaccagcaccgcgtatatggaactgagcagcctgcgtagcgaagatacggccgtgtattattgcgcgcgttctaagaagggtatgtatggtggttggacttatcctcttatgatgtttgatctttggggccaaggcaccctggtgacggttagctca

SEQ ID NO: 136 - DNA, 324 bp, Homo sapiens
gagatcgtgctgacccagagccccgccaccctgagcctgagccccggcgagcgcgccaccctgagctgccgcgccagccagagcgtgagcagcaactacctggcctggtaccagcagaagcccggccaggccccccgcctgctgatctactacgccagccgccgcgccaccggcgtgcccgcccgcttcagcggcagcggcagcggcaccgacttcaccctgaccatcagcagcctggagcccgaggacttcgccgtgtactactgccagcagaccagcaacacccccttcaccttcggccagggcaccaaggtggagatcaag

SEQ ID NO: 137 - DNA, 324 bp, Homo sapiens
gaaattgtgttgacacagtctccagccaccctgtctttgtctccaggggaaagagccaccctctcctgcagggccagtcagagtgttagcagcaactacttagcctggtaccaacagaaacctggccaggctcccaggctcctcatctattacgcatcccgcagggccactggcgtgccagccaggttcagtggcagtgggtctgggacagacttcactctcaccatcagcagcctagagcctgaagattttgcagtttattactgtcagcagacttctaatactccttttacctttggccagggtacgaaagttgaaattaaa

SEQ ID NO: 138 - DNA, 324 bp, Homo sapiens
gagatcgtgctgacccagagcccggcgaccctgagcctgtctccgggcgaacgtgcgaccctgagctgcagagcgagccagtctgtttcttctaattatctggcttggtaccagcagaaaccaggtcaagcaccgcgtctattaatttattatgcttctcgtcgtgcaactggggtcccggcgcgttttagcggctctggatccggcacggattttaccctgaccattagcagcctggaacctgaagactttgcggtgtattattgccagcagacttctaatactccttttacctttggccagggtacgaaagttgaaattaaa

SEQ ID NO: 139 - DNA, 351 bp, Homo sapiens
gaggtgcagctggtgcagtctggagcagaggtgaaaaagcccggggagtctctgaagatctcctgtaagggttctggatacagctttagcaactactggatcggctgggtgcgccagatgcccgggaaaggcctggagtggatggggatcatcgaccctagcaactcttacaccagatacagcccgtccttccaaggccaggtcaccatctcagccgacaagtccatcagcaccgcctacctgcagtggagcagcctgaaggcctcggacaccgccatgtattactgtgcgagatggtactacaagcccttcgacgtgtggggccagggcaccctggtgaccgtgagcagc

SEQ ID NO: 140 - DNA, 351 bp, Homo sapiens
gaggtgcagctggtgcagagcggcgccgaggtgaagaagcccggcgagagcctgaagatcagctgcaagggcagcggctacagcttcagcaactactggatcggctgggtgcgccagatgcccggcaagggcctggagtggatgggcatcatcgaccccagcaacagctacacccgctacagccccagcttccagggccaggtgaccatcagcgccgacaagagcatcagcaccgcctacctgcagtggagcagcctgaaggccagcgacaccgccatgtactactgcgcccgctggtactacaagcccttcgacgtgtggggccagggcaccctggtgaccgtgagcagc

SEQ ID NO: 141 - DNA, 351 bp, Homo sapiens
gaggtgcaattggttcagagcggcgcggaagtgaaaaaaccgggcgaaagcctgaaaattagctgcaaaggttccggatattccttttctaattattggattggttgggtgcgccagatgcctgggaagggtctcgagtggatgggcattatcgatccgtctaatagctatacccgctattctccgagctttcagggccaggtgaccattagcgcggataaaagcattagcaccgcgtatcttcaatggagcagcctgaaagcgagcgatacggccatgtattattgcgcgcgttggtattataagccttttgatgtttggggccaaggcaccctggtgacggttagctca

SEQ ID NO: 142 - DNA, 336 bp, Homo sapiens
cagtctgtgctgacgcagccgccctcagtgtctggggccccagggcagagggtcaccatctcctgcactgggagcagctccaacatcgggagcggttatgatgtacactggtaccagcagcttccaggaacagcccccaaactcctcatctatggtaacagcaagcggccctcaggggtccctgaccgattctctggctccaagtctggcacctcagcctccctggccatcactgggctccagagcgaggatgaggctgattattactgcgccagctggaccgacggcctgagcctggtggtgttcggcggcggcaccaagctgaccgtgctgggc

SEQ ID NO: 143 - DNA, 336 bp, Homo sapiens
cagagcgtgctgacccagccccccagcgtgagcggcgcccccggccagcgcgtgaccatcagctgcaccggcagcagcagcaacatcggcagcggctacgacgtgcactggtaccagcagctgcccggcaccgcccccaagctgctgatctacggcaacagcaagcgccccagcggcgtgcccgaccgcttcagcggcagcaagagcggcaccagcgccagcctggccatcaccggcctccagagcgaggacgaggccgactactactgtgccagctggaccgacggcctgagcctggtggtgttcggcggcggcaccaagctgaccgtgctgggc

SEQ ID NO: 144 - DNA, 336 bp, Homo sapiens
cagagcgtgctgacccagccgccttcagtgagtggcgcaccaggtcagcgtgtgaccatctcgtgtacgggcagcagcagcaacattggttctggttatgatgtgcattggtaccagcagttgcccgggacggcgccgaaacttctgatttatggtaattctaagcgtccctcaggcgtgccggatcgttttagcggatccaaaagcggcaccagcgcgagccttgcgattacgggcctgcaaagcgaagacgaagcggattattattgcgcttcttggactgatggtctttctcttgttgtgtttggcggcggcacgaagttaaccgttcttggc

SEQ ID NO: 145 - protein, 189 aa, Homo sapiens [sequence omitted]

SEQ ID NO: 146 - protein, 19 aa, Homo sapiens
NIEHKYLGYATSYAASVKG

SEQ ID NO: 147 - protein, 123 aa, Homo sapiens
QVQLVESGGGLVQPGGSLRLSCAASGFTFSSFGMSWVRQAPGKGLEWVSNIEHKYLGYATSYAASVKGRFTISRDNSKNTLYLQMNSLRAEDTAVYYCARYWGTPYLMQFDNWGQGTLVTVSS

SEQ ID NO: 148 - protein, 12 aa, Homo sapiens
HQGLIFYEKLLG